European Patent Specification EP 3 469 102 B1, published January 25, 2023. Title: COMPOSITIONS AND METHODS FOR THE DETECTION OF HEPATITIS C VIRUS GENOTYPE 3. Applicant: Roche Diagnostics GmbH F. Hoffmann-La Roche AG Roche Molecular Systems, Inc. The sequence listing filed with the application follows.

SEQUENCE LISTING (4 sequences)

SEQ ID NO: 1 - DNA, 18 bp, Artificial Sequence
  Forward Primer
  modified_base (18)..(18): t-Butyl benzyl-dA
cttctgtcttcacgcgga

SEQ ID NO: 2 - DNA, 17 bp, Artificial Sequence
  Probe
  modified_base (2)..(2): 5-propynyl dC
  modified_base (6)..(6): 5-propynyl dU
  modified_base (8)..(8): 5-propynyl dU
  modified_base (9)..(9): 5-propynyl dC
  modified_base (11)..(11): 5-propynyl dU
  modified_base (13)..(13): 5-propynyl dC
  modified_base (16)..(17): 5-propynyl dC
acgagugucgugcagcc

SEQ ID NO: 3 - DNA, 24 bp, Artificial Sequence
  Reverse Primer
  modified_base (24)..(24): 2'-O-Methyl ribo U
ctcgcaagcaccctatcaggcagu

SEQ ID NO: 4 - DNA, 17 bp, Artificial Sequence
  Reverse Primer
  modified_base (17)..(17): t-Butyl benzyl-dA
cctttcgcgacccaaca